European Patent Specification EP 3 669 005 B1, published March 4, 2026. Title: ERGIC1 as epigenetic marker for the identification of immune cells, in particular monocytic myeloid-derived suppressor cells (mMDSCs). Applicant: Epiontis GmbH. The sequence listing filed with the application follows.

SEQUENCE LISTING (11 sequences)

SEQ ID NO: 1 - DNA, 455 bp, Homo sapiens
gagggaatgagtaggtgaacaaacgagtgagtttttcgcctcactccctggcactcggcaccgagggctccgacaggctggtggccagggctgaccagccagagtttcatctaaaagcctcgatggctatttttgggacaaatgacccaccacttccaatgacttgctccgaaatggcatctaatttcattaagccttggaaacagtgacatcacaagtgcctgcccggtagccgcccacatatggcgaaccacagagtgatccgagattcgtctgcaagaacaggggagaactaaggtcccaagcagcaaaagttaaaatagcaaagctgaggcattctgctatgaaaagaaattacagatgaaatccattagtcagacatttccagcggcagtttccttgcttgggagcaggggaagacgtgtttattcggggttgggctctgcagccattcc

SEQ ID NO: 2 - DNA, 455 bp, Homo sapiens
aaaaaaataaataaataaacaaacgaataaatttttcgcctcactccctaacactcgacaccgaaaactccgacaaactaataaccaaaactaaccaaccaaaatttcatctaaaaacctcgataactatttttaaaacaaataacccaccacttccaataacttactccgaaataacatctaatttcattaaaccttaaaaacaataacatcacaaatacctacccgataaccgcccacatataacgaaccacaaaataatccgaaattcgtctacaaaaacaaaaaaaaactaaaatcccaaacaacaaaaattaaaataacaaaactaaaacattctactataaaaaaaaattacaaataaaatccattaatcaaacatttccaacgacaatttccttacttaaaaacaaaaaaaaacgtatttattcgaaattaaactctacaaccattcc

SEQ ID NO: 3 - DNA, 455 bp, Homo sapiens
aaaaaaataaataaataaacaaacaaataaatttttcacctcactccctaacactcaacaccaaaaactccaacaaactaataaccaaaactaaccaaccaaaatttcatctaaaaacctcaataactatttttaaaacaaataacccaccacttccaataacttactccaaaataacatctaatttcattaaaccttaaaaacaataacatcacaaatacctaccccataaccacccacatataacaaaccacaaaataatccaaaattcatctacaaaaacaaaaaaaaactaaaatcccaaacaacaaaaattaaaataacaaaactaaaacattctactataaaaaaaaattacaaataaaatccattaatcaaacatttccaacaacaatttccttacttaaaaacaaaaaaaaacatatttattcaaaattaaactctacaaccattcc

SEQ ID NO: 4 - DNA, 22 bp, Homo sapiens
gagggaatgagtaggtgaataa

SEQ ID NO: 5 - DNA, 22 bp, Homo sapiens
aaaataactacaaaacccaacc

SEQ ID NO: 6 - DNA, 18 bp, Homo sapiens
ccctaacactcaacacca

SEQ ID NO: 7 - DNA, 28 bp, Homo sapiens
gggttatttgttttaaaaatagttattg

SEQ ID NO: 8 - DNA, 28 bp, Homo sapiens
tggttattagtttgttggagtttttggt

SEQ ID NO: 9 - DNA, 18 bp, Homo sapiens
ccctaacactcgacaccg

SEQ ID NO: 10 - DNA, 27 bp, Homo sapiens
gggttatttgttttaaaaatagttatc

SEQ ID NO: 11 - DNA, 30 bp, Homo sapiens
ttttggttattagtttgtcggagttttcgg